European Patent Application EP 4 464 332 A1, published November 20, 2024. Title: COMPOSITION FOR IMPROVING THE SOLUBILITY OF A PROTEIN OR PEPTIDE BY USING IMMUNOGLOBULIN FC FRAGMENT LINKAGE. Applicant: HANMI PHARM. CO., LTD. Application EP 24182153.7, filed March 31, 2015. The sequence listing filed with the application follows.

SEQUENCE LISTING (52 sequences)

SEQ ID NO: 1 - protein, 21 aa, synthetic construct
  REGION 1..21: note = Insulin alpha chain
GIVEQCCTSICSLYQLENYCN

SEQ ID NO: 2 - protein, 30 aa, synthetic construct
  REGION 1..30: note = Insulin beta chain
FVNQHLCGSHLVEALYLVCGERGFFYTPKT

SEQ ID NO: 3 - protein, 37 aa, Homo sapiens
HSQGTFTSDYSKYLDSRRAQDFVQWLMNTKRNRNNIA

SEQ ID NO: 4 - protein, 37 aa, synthetic construct
  VARIANT 1: note = Xaa is 4-imidazoacetyl.
XSQGTFTSDYSKYLDEEAVRLFIEWLMNTKRNRNNIA

SEQ ID NO: 5 - protein, 39 aa, synthetic construct
  VARIANT 1: note = Xaa is 4-imidazoacetyl.
XSQGTFTSDYSKYLDERRAQDFVAWLKNTGPSSGAPPPS

SEQ ID NO: 6 - protein, 39 aa, synthetic construct
  VARIANT 1: note = Xaa is 4-imidazoacetyl.
XGQGTFTSDYSRYLEEEAVRLFIEWLKNGGPSSGAPPPS

SEQ ID NO: 7 - protein, 39 aa, synthetic construct
  VARIANT 1: note = Xaa is 4-imidazoacetyl.
XGQGTFTSDYSRQMEEEAVRLFIEWLKNGGPSSGAPPPS

SEQ ID NO: 8 - protein, 42 aa, synthetic construct
  VARIANT 1: note = Xaa is 4-imidazoacetyl.
XGEGTFTSDLSRQMEEEAVRLFIEWAAHSQGTFTSDYSKYLD

SEQ ID NO: 9 - protein, 30 aa, synthetic construct
  VARIANT 1: note = Xaa is 4-imidazoacetyl.
XSQGTFTSDYSRYLDEEAVRLFIEWLMNTK

SEQ ID NO: 10 - protein, 29 aa, synthetic construct
  VARIANT 1: note = Xaa is 4-imidazoacetyl.
XSQGTFTSDLSRQLEEEAVRLFIEWLMNK

SEQ ID NO: 11 - protein, 37 aa, synthetic construct
  VARIANT 1: note = Xaa is 4-imidazoacetyl.
  VARIANT 20: note = Xaa = alpha-methyl-glutamic acid
XGQGTFTSDYSRYLDEEAVXLFIEWLMNTKRNRNNIA

SEQ ID NO: 12 - protein, 40 aa, synthetic construct
  VARIANT 1: note = Xaa is 4-imidazoacetyl.
XSQGTFTSDYSRQMEEEAVRLFIEWLMNGGPSSGAPPPSK

SEQ ID NO: 13 - protein, 43 aa, synthetic construct
  VARIANT 1: note = Xaa is 4-imidazoacetyl.
XGEGTFTSDLSRQMEEEAVRLFIEWAAHSQGTFTSDYSRYLDK

SEQ ID NO: 14 - protein, 38 aa, synthetic construct
  VARIANT 1: note = Xaa is 4-imidazoacetyl.
XSQGTFTSDYSRYLDGGGHGEGTFTSDLSKQMEEEAVK

SEQ ID NO: 15 - protein, 30 aa, synthetic construct
  VARIANT 1: note = Xaa is 4-imidazoacetyl.
  VARIANT 16: note = Xaa = alpha-methyl-glutamic acid
  VARIANT 20: note = Xaa = alpha-methyl-glutamic acid
XSQGTFTSDYSRYLDXEAVXLFIEWLMNTK

SEQ ID NO: 16 - protein, 37 aa, synthetic construct
  VARIANT 1: note = Xaa is 4-imidazoacetyl.
  VARIANT 20: note = Xaa = alpha-methyl-glutamic acid
  VARIANT 24: note = Xaa = alpha-methyl-glutamic acid
XGQGTFTSDYSRYLDEEAVXLFIXWLMNTKRNRNNIA

SEQ ID NO: 17 - protein, 37 aa, synthetic construct
  VARIANT 1: note = Xaa is 4-imidazoacetyl.
  VARIANT 24: note = Xaa = alpha-methyl-glutamic acid
XGQGTFTSDYSRYLDEEAVRLFIXWLMNTKRNRNNIA

SEQ ID NO: 18 - protein, 34 aa, synthetic construct
  VARIANT 1: note = Xaa is 4-imidazoacetyl.
XSQGTFTSDLSRQLEGGGHSQGTFTSDLSRQLEK

SEQ ID NO: 19 - protein, 37 aa, synthetic construct
  VARIANT 1: note = Xaa is 4-imidazoacetyl.
XSQGTFTSDYSRYLDEEAVRLFIEWIRNTKRNRNNIA

SEQ ID NO: 20 - protein, 40 aa, synthetic construct
  VARIANT 1: note = Xaa is 4-imidazoacetyl.
XSQGTFTSDYSRYLDEEAVRLFIEWIRNGGPSSGAPPPSK

SEQ ID NO: 21 - protein, 37 aa, synthetic construct
  VARIANT 1: note = Xaa is 4-imidazoacetyl.
XSQGTFTSDYSRYLDEEAVKLFIEWIRNTKRNRNNIA

SEQ ID NO: 22 - protein, 40 aa, synthetic construct
  VARIANT 1: note = Xaa is 4-imidazoacetyl.
XSQGTFTSDYSRYLDEEAVKLFIEWIRNGGPSSGAPPPSK

SEQ ID NO: 23 - protein, 37 aa, synthetic construct
  VARIANT 1: note = Xaa is 4-imidazoacetyl.
XSQGTFTSDYSRQLEEEAVRLFIEWVRNTKRNRNNIA

SEQ ID NO: 24 - protein, 30 aa, synthetic construct
  VARIANT 1: note = Xaa is desamino-histidyl.
XSQGTFTSDYSKYLDEKRAKEFVQWLMNTK

SEQ ID NO: 25 - protein, 29 aa, synthetic construct
  VARIANT 2: note = Xaa = aminoisobutyric acid
HXQGTFTSDYSKYLDEKRAKEFVCWLMNT

SEQ ID NO: 26 - protein, 30 aa, synthetic construct
  VARIANT 2: note = Xaa = aminoisobutyric acid
HXQGTFTSDYSKYLDEKRAKEFVQWLMNTC

SEQ ID NO: 27 - protein, 30 aa, synthetic construct; identical to SEQ ID NO: 26
  VARIANT 2: note = Xaa = aminoisobutyric acid

SEQ ID NO: 28 - protein, 30 aa, synthetic construct; identical to SEQ ID NO: 26
  VARIANT 2: note = Xaa = aminoisobutyric acid

SEQ ID NO: 29 - protein, 29 aa, synthetic construct
  REGION 1..29: note = oxyntomodulin derivative
  VARIANT 2: note = Xaa = aminoisobutyric acid
HXQGTFTSDYSKYLDEQAAKEFICWLMNT

SEQ ID NO: 30 - protein, 29 aa, synthetic construct
  VARIANT 2: note = Xaa = aminoisobutyric acid
HXQGTFTSDYSKYLDEKRAKEFVQWLMNT

SEQ ID NO: 31 - protein, 37 aa, synthetic construct
  VARIANT 2: note = Xaa is d-serine.
HXQGTFTSDYSKYLDSRRAQDFVQWLMNTKRNRNNIA

SEQ ID NO: 32 - protein, 37 aa, synthetic construct
  VARIANT 1: note = Xaa is 4-imidazoacetyl.
XSQGTFTSDYSKYLDSRRAQDFVQWLMNTKRNRNNIA

SEQ ID NO: 33 - protein, 37 aa, synthetic construct
  VARIANT 1: note = Xaa is 4-imidazoacetyl.
  VARIANT 2: note = Xaa is d-serine.
XXQGTFTSDYSKYLDSRRAQDFVQWLMNTKRNRNNIA

SEQ ID NO: 34 - protein, 30 aa, synthetic construct
  REGION 1..30: note = oxyntomodulin derivative
  VARIANT 1: note = Xaa is 4-imidazoacetyl.
  VARIANT 2: note = Xaa = aminoisobutyric acid
XXQGTFTSDYSKYLDEKRAKEFVQWLMNTC

SEQ ID NO: 35 - protein, 30 aa, synthetic construct
  REGION 1..30: note = oxyntomodulin derivative
  VARIANT 2: note = Xaa = aminoisobutyric acid
HXQGTFTSDYAKYLDEKRAKEFVQWLMNTC

SEQ ID NO: 36 - protein, 30 aa, synthetic construct
  REGION 1..30: note = oxyntomodulin derivative
  VARIANT 2: note = Xaa = aminoisobutyric acid
YXQGTFTSDYSKYLDEKRAKEFVQWLMNTC

SEQ ID NO: 37 - protein, 8 aa, synthetic construct
  REGION 1..8: note = group R2
KRNRNNIA

SEQ ID NO: 38 - protein, 10 aa, synthetic construct
  REGION 1..10: note = group R2
GPSSGAPPPS

SEQ ID NO: 39 - protein, 11 aa, synthetic construct
  REGION 1..11: note = group R2
GPSSGAPPPSK

SEQ ID NO: 40 - protein, 15 aa, synthetic construct
  REGION 1..15: note = group R2
HSQGTFTSDYSKYLD

SEQ ID NO: 41 - protein, 16 aa, synthetic construct
  REGION 1..16: note = group R2
HSQGTFTSDYSRYLDK

SEQ ID NO: 42 - protein, 20 aa, synthetic construct
  REGION 1..20: note = group R2
HGEGTFTSDLSKQMEEEAVK

SEQ ID NO: 43 - protein, 28 aa, synthetic construct
  REGION 1..28: note = group A or B
SQGTFTSDYSKYLDSRRAQDFVQWLMNT

SEQ ID NO: 44 - protein, 28 aa, synthetic construct
  REGION 1..28: note = group A or B
SQGTFTSDYSKYLDEEAVRLFIEWLMNT

SEQ ID NO: 45 - protein, 28 aa, synthetic construct
  REGION 1..28: note = group A or B
SQGTFTSDYSKYLDERRAQDFVAWLKNT

SEQ ID NO: 46 - protein, 28 aa, synthetic construct
  REGION 1..28: note = group A or B
GQGTFTSDYSRYLEEEAVRLFIEWLKNG

SEQ ID NO: 47 - protein, 28 aa, synthetic construct
  REGION 1..28: note = group A or B
GQGTFTSDYSRQMEEEAVRLFIEWLKNG

SEQ ID NO: 48 - protein, 26 aa, synthetic construct
  REGION 1..26: note = group A or B
GEGTFTSDLSRQMEEEAVRLFIEWAA

SEQ ID NO: 49 - protein, 28 aa, synthetic construct
  REGION 1..28: note = group A or B
SQGTFTSDYSRQMEEEAVRLFIEWLMNG

SEQ ID NO: 50 - protein, 24 aa, synthetic construct
  REGION 1..24: note = group B
GEGTFTSDLSRQMEEEAVRLFIEW

SEQ ID NO: 51 - protein, 14 aa, synthetic construct
  REGION 1..14: note = group B
SQGTFTSDYSRYLD

SEQ ID NO: 52 - protein, 29 aa, synthetic construct
  REGION 1..29: note = Glucagon
HSQGTFTSDYSKYLDSRRAQDFVQWLMNT